European Patent Application EP 4 710 944 A1, published March 18, 2026. Title: ANTI-PDL1 ANTIBODY-DRUG CONJUGATE AND USE. Applicant: SHANGHAI HENLIUS BIOTECH, INC. The sequence listing filed with the application follows.

SEQUENCE LISTING (16 sequences)

SEQ ID NO: 1 - protein, 5 aa, synthetic construct
  source 1..5: note = MAB20 HC CDR1
SYTMN

SEQ ID NO: 2 - protein, 17 aa, synthetic construct
  source 1..17: note = MAB20 HC CDR2
SISSGSDYLYYADSVKG

SEQ ID NO: 3 - protein, 14 aa, synthetic construct
  source 1..14: note = MAB20 HC CDR3
NELRWYPQAGAFDR

SEQ ID NO: 4 - protein, 13 aa, synthetic construct
  source 1..13: note = MAB20 LC CDR1
SGSSSYIESSYVG

SEQ ID NO: 5 - protein, 7 aa, synthetic construct
  source 1..7: note = MAB20 LC CDR2
DDDMRPS

SEQ ID NO: 6 - protein, 10 aa, synthetic construct
  source 1..10: note = MAB20 LC CDR3
EIWRSGLGGV

SEQ ID NO: 7 - protein, 123 aa, synthetic construct
  source 1..123: note = MAB20 VH
EVQLVQSGGGLVKPGGSLRLSCAASGFTFSSYTMNWVRQAPGKGLEWVSSISSGSDYLYYADSVKGRFTISRDNAKNSLYLQMNSLRAEDTAVYYCARNELRWYPQAGAFDRWGQGTMVTVSS

SEQ ID NO: 8 - protein, 112 aa, synthetic construct
  source 1..112: note = MAB20 VL
QSVVTQPPSMSAAPGQRVTISCSGSSSYIESSYVGWYQQLPGTAPRLLIYDDDMRPSGIPDRFSGSKSGTSATLAITGLQTGDEADYYCEIWRSGLGGVFGGGTKLTVLSQP

SEQ ID NO: 9 - protein, 453 aa, synthetic construct
  source 1..453: note = MAB20 HC
EVQLVQSGGGLVKPGGSLRLSCAASGFTFSSYTMNWVRQAPGKGLEWVSSISSGSDYLYYADSVKGRFTISRDNAKNSLYLQMNSLRAEDTAVYYCARNELRWYPQAGAFDRWGQGTMVTVSSASTKGPSVFPLAPSSKSTSGGTAALGCLVKDYFPEPVTVSWNSGALTSGVHTFPAVLQSSGLYSLSSVVTVPSSSLGTQTYICNVNHKPSNTKVDKKVEPKSCDKTHTCPPCPAPELLGGPSVFLFPPKPKDTLMISRTPEVTCVVVDVSHEDPEVKFNWYVDGVEVHNAKTKPREEQYASTYRVVSVLTVLHQDWLNGKEYKCKVSNKALPAPIEKTISKAKGQPREPQVYTLPPSREEMTKNQVSLTCLVKGFYPSDIAVEWESNGQPENNYKTTPPVLDSDGSFFLYSKLTVDKSRWQQGNVFSCSVMHEALHNHYTQKSLSLSPGK

SEQ ID NO: 10 - protein, 214 aa, synthetic construct
  source 1..214: note = MAB20 LC
QSVVTQPPSMSAAPGQRVTISCSGSSSYIESSYVGWYQQLPGTAPRLLIYDDDMRPSGIPDRFSGSKSGTSATLAITGLQTGDEADYYCEIWRSGLGGVFGGGTKLTVLSQPKAAPSVTLFPPSSEELQANKATLVCLISDFYPGAVTVAWKADSSPVKAGVETTTPSKQSNNKYAASSYLSLTPEQWKSHKSYSCQVTHEGSTVERTVALTEC

SEQ ID NO: 11 - protein, 220 aa, synthetic construct
  source 1..220: note = Human PDL1 ECD
FTVTVPKDLYVVEYGSNMTIECKFPVEKQLDLAALIVYWEMEDKNIIQFVHGEEDLKVQHSSYRQRARLLKDQLSLGNAALQITDVKLQDAGVYRCMISYGGADYKRITVKVNAPYNKINQRILVVDPVTSEHELTCQAEGYPKAEVIWTSSDHQVLSGKTTTTNSKREEKLFNVTSTLRINTTTNEIFYCTFRRLDPEENHTAELVIPELPLAHPPNER

SEQ ID NO: 12 - protein, 222 aa, synthetic construct
  source 1..222: note = Monkey PDL1 ECD
FTVTVPKDLYVVEYGSNMTIECKFPVEKQLDLTSLIVYWEMEDKNIIQFVHGEEDLKVQHSNYRQRAQLLKDQLSLGNAALRITDVKLQDAGVYRCMISYGGADYKRITVKVNAPYNKINQRILVVDPVTSEHELTCQAEGYPKAEVIWTSSDHQVLSGKTTTTNSKREEKLLNVTSTLRINTTANEIFYCIFRRLDPEENHTAELVIPELPLALPPNERTH

SEQ ID NO: 13 - protein, 221 aa, synthetic construct
  source 1..221: note = Rat PDL1 ECD
FTITAPKDLYVVEYGSNVTMECRFPVEQKLDLLALVVYWEKEDKEVIQFVEGEEDLKPQHSSFRGRAFLPKDQLLKGNAVLQITDVKLQDAGVYCCMISYGGADYKRITLKVNAPYRKINQRISMDPATSEHELMCQAEGYPEAEVIWTNSDHQSLSGETTVTTSQTEEKLLNVTSVLRVNATANDVFHCTFWRVHSGENHTAELIIPELPVPRLPHNRTH

SEQ ID NO: 14 - protein, 221 aa, synthetic construct
  source 1..221: note = Mice PDL1 ECD
FTITAPKDLYVVEYGSNVTMECRFPVERELDLLALVVYWEKEDEQVIQFVAGEEDLKPQHSNFRGRASLPKDQLLKGNAALQITDVKLQDAGVYCCIISYGGADYKRITLKVNAPYRKINQRISVDPATSEHELICQAEGYPEAEVIWTNSDHQPVSGKRSVTTSRTEGMLLNVTSSLRVNATANDVFYCTFWRSQPGQNHTAELIIPELPATHPPQNRTH

SEQ ID NO: 15 - protein, 453 aa, synthetic construct
  source 1..453: note = HC of SGN-PDL1V antibody
QVQLVQSGAEVKKPGSSVKVSCKTSGDTFSTAAISWVRQAPGQGLEWMGGIIPIFGKAHYAQKFQGRVTITADESTSTAYMELSSLRSEDTAVYFCARKFHFVSGSPFGMDVWGQGTTVTVSSASTKGPSVFPLAPSSKSTSGGTAALGCLVKDYFPEPVTVSWNSGALTSGVHTFPAVLQSSGLYSLSSVVTVPSSSLGTQTYICNVNHKPSNTKVDKKVEPKSCDKTHTCPPCPAPEAAGGPSVFLFPPKPKDTLMISRTPEVTCVVVDVSHEDPEVKFNWYVDGVEVHNAKTKPREEQYNSTYRVVSVLTVLHQDWLNGKEYKCKVSNKALPAPIEKTISKAKGQPREPQVYTLPPSRDELTKNQVSLTCLVKGFYPSDIAVEWESNGQPENNYKTTPPVLDSDGSFFLYSKLTVDKSRWQQGNVFSCSVMHEALHNHYTQKSLSLSPGK

SEQ ID NO: 16 - protein, 213 aa, synthetic construct
  source 1..213: note = LC of SGN-PDL1V antibody
EIVLTQSPATLSLSPGERATLSCRASQSVSSYLAWYQQKPGQAPRLLIYDASNRATGIPARFSGSGSGTDFTLTISSLEPEDFAVYYCQQRSNWPTFGQGTKVEIKRTVAAPSVFIFPPSDEQLKSGTASVVCLLNNFYPREAKVQWKVDNALQSGNSQESVTEQDSKDSTYSLSSTLTLSKADYEKHKVYACEVTHQGLSSPVTKSFNRGEC